European Patent Specification EP 2 966 167 B1, published October 29, 2025. Title: PRSV resistance Cucumis sativus L. and production method of PRSV and ZYMV resistance Cucumis sativus L. Applicant: Takii & Co.,Ltd. The sequence listing filed with the application follows.

SEQUENCE LISTING (6 sequences)

SEQ ID NO: 1 - DNA, 404 bp, Cucumis sativus
agcaatttcaaggagcaagctattaaatacgtgaagcaggcggtacatgaagataatgctggcaattacgcaaaagcctttccgctgtatatgaacgccttggagtacttcaaaacttatttgaagtatcagaaaaatcccaagatcaaggaagctattacccagaaattcaccgagtatttgcgccgggctgaggagatacgtgctgttttggatgatggcggtcctggtccggcttccaatggagatgcagctgttgcaactaaacccaagacgaaacctaaggatggagaaggaggagatggagaggatccaggacaggctaagttacgggctggtcttaattccgcaatcataagggagaaaccggatgttaagtggaacgatgttgctggattggagag

SEQ ID NO: 2 - DNA, 404 bp, Cucumis sativus
agcaatttcaaggagcaagctattgaatacgtgaagcaggcggtacatgaagataatgctggcaattacgcaaaagcctctccgctgtatataaacgccttggagtacttcaaaactcatttgaagtatgagaaaaatcccaagatcaaggaagctattacccagaaattcaccgagtatttgcgccgggctgaggagatacgtgctgttttggatgatggcggtcctggtccggcttccaatggagatgcagctgttgcaactaaacccaagacgaaacctaaggatggagaaggaggagatggaaaggatccagaacaggctaagttacgggctggtcttaattccgcaatcataagggagaaaccggatgttaagtggaacgatgttgctggattggagag

SEQ ID NO: 3 - DNA, 404 bp, Cucumis sativus
agcaatttcaaggagcaagctattgaatacgtgaagcaggcggtacatgaagataatgctggcaattacgcaaaagcctctccgctgtatataaacgccttggagtacttcaaaactcatttgaagtatgagaaaaatcccaagatcaaggaagctattacccagaaattcaccgagtatttgcgccgggctgaggagatacgtgctgttttggatgatggcggtcctggtccggcttccaatggagatgcagctgttgcaactaaacccaagacgaaacctaaggatggagaaggaggagatggagaggatccagaacaggctaagttacgggctggtcttaattccgcaatcataagggagaaaccggatgttaagtggaacgatgttgctggattggagag

SEQ ID NO: 4 - DNA, 404 bp, Cucumis sativus
  misc_feature (25)..(25): n is a, c, g, or t
  misc_feature (80)..(80): n is a, c, g, or t
  misc_feature (93)..(93): n is a, c, g, or t
  misc_feature (118)..(118): n is a, c, g, or t
  misc_feature (130)..(130): n is a, c, g, or t
  misc_feature (307)..(307): n is a, c, g, or t
  misc_feature (317)..(317): n is a, c, g, or t
agcaatttcaaggagcaagctattnaatacgtgaagcaggcggtacatgaagataatgctggcaattacgcaaaagcctntccgctgtatatnaacgccttggagtacttcaaaactnatttgaagtatnagaaaaatcccaagatcaaggaagctattacccagaaattcaccgagtatttgcgccgggctgaggagatacgtgctgttttggatgatggcggtcctggtccggcttccaatggagatgcagctgttgcaactaaacccaagacgaaacctaaggatggagaaggaggagatgganaggatccagnacaggctaagttacgggctggtcttaattccgcaatcataagggagaaaccggatgttaagtggaacgatgttgctggattggagag

SEQ ID NO: 5 - DNA, 20 bp, Artificial Sequence
  primer
agcaatttcaaggagcaagc

SEQ ID NO: 6 - DNA, 19 bp, Artificial Sequence
  primer
ctctccaatccagcaacat